European Patent Specification EP 3 878 975 B1, published June 3, 2026. Title: PHASE-PROTECTING REAGENT FLOW ORDERINGS FOR USE IN SEQUENCING-BY-SYNTHESIS. Applicant: LIFE TECHNOLOGIES CORPORATION. Application PCT/US2012/032418. The sequence listing filed with the application follows.

SEQUENCE LISTING (21 sequences)

SEQ ID NO: 1 - DNA, 22 bp, Artificial Sequence
  Exemplary Strand
tagcactacggaacgtgaaggt

SEQ ID NO: 2 - DNA, 40 bp, Artificial Sequence
  Ordering of Nucleotide Species Flows
tacgtacgtacgtacgtacgtacatacgcacgtgcgtatg

SEQ ID NO: 3 - DNA, 16 bp, Artificial Sequence
  Ordering of Nucleotide Species Flows
tacgtacgtctgagca

SEQ ID NO: 4 - DNA, 104 bp, Artificial Sequence
  Ordering of Nucleotide Species Flows
tacgtacgtagcttgacgtacgtcatgcatcgatcagctaagctgacgtagctagcatcgatccagtcatgactgacgtagctgactggatcagtcatgcatcg

SEQ ID NO: 5 - DNA, 100 bp, Artificial Sequence
  Ordering of Nucleotide Species Flows
tacgtacgtagctgacgtacgtcatgcatcgatcagctagctgacgtagctagcatcgatcagtcatgactgacgtagctgactgatcagtcatgcatcg

SEQ ID NO: 6 - DNA, 40 bp, Artificial Sequence; identical to SEQ ID NO: 2
  Ordering of Nucleotide Species Flows

SEQ ID NO: 7 - DNA, 32 bp, Artificial Sequence
  Ordering of Nucleotide Species Flows
tacgtacgtctgagcatcgatcgatgtacagc

SEQ ID NO: 8 - DNA, 192 bp, Artificial Sequence
  Ordering of Nucleotide Species Flows
tacgtacgtctgagcatcgatcgatgtacagctgactgactatcgcagagctagctacatgtcgactgactgatagcgtcatgcatgcagactcgtcgtacgtactcagatgctagctagcacgtgatcagtcagtcgctatgagtcagtcagcgatactgcatgcatgagtctacgatcgatcgtgcacta

SEQ ID NO: 9 - DNA, 64 bp, Artificial Sequence
  Ordering of Nucleotide Species Flows
cttgcttacaactctcatatcggtatcctgtggaaactccgttatcagcatcctctcatgttag

SEQ ID NO: 10 - DNA, 36 bp, Artificial Sequence
  Ordering of Nucleotide Species Flows
tacactctagtatagagtcgtgtctcgacgcgagac

SEQ ID NO: 11 - DNA, 20 bp, Artificial Sequence
  Ordering of Nucleotide Species Flows
tactcagtatgcagactgcg

SEQ ID NO: 12 - DNA, 52 bp, Artificial Sequence
  Ordering of Nucleotide Species Flows
tacgtacgtactcagctagctagtatgcatgcatgcagactgactgactgcg

SEQ ID NO: 13 - DNA, 40 bp, Artificial Sequence
  Ordering of Nucleotide Species Flows
tacgtacgtactcagctagtatgcatgcagactgactgcg

SEQ ID NO: 14 - DNA, 44 bp, Artificial Sequence
  Ordering of Nucleotide Species Flows
tacgtacgttactcagctaagtatgcatggcagactgacctgcg

SEQ ID NO: 15 - DNA, 12 bp, Artificial Sequence
  Ordering of Nucleotide Species Flows
tacgtctgagca

SEQ ID NO: 16 - DNA, 40 bp, Artificial Sequence
  Ordering of Nucleotide Species Flows
tacgtacgtacgtacgtacgtacgtacgcacgtgcgtatg

SEQ ID NO: 17 - DNA, 40 bp, Artificial Sequence; identical to SEQ ID NO: 13
  Ordering of Nucleotide Species Flows

SEQ ID NO: 18 - DNA, 12 bp, Artificial Sequence
  Ordering of Nucleotide Species Flows
tctagactcgag

SEQ ID NO: 19 - DNA, 12 bp, Artificial Sequence
  Ordering of Nucleotide Species Flows
tcgatgtacagc

SEQ ID NO: 20 - DNA, 20 bp, Artificial Sequence
  Ordering of Nucleotide Species Flows
tacatacgcacgtgcgtatg

SEQ ID NO: 21 - DNA, 40 bp, Artificial Sequence; identical to SEQ ID NO: 2
  Ordering of Nucleotide Species Flows